European Patent Application EP 4 512 911 A1, published February 26, 2025. Title: METHOD FOR REGULATING AND CONTROLLING MALT PYF ON BASIS OF GENE EXPRESSION IN MALTING PROCESS AND USE THEREOF. Applicant: TSINGTAO BREWERY CO., LTD. Application EP 23854564.4, filed November 6, 2023. The sequence listing filed with the application follows.

SEQUENCE LISTING (26 sequences)

SEQ ID NO: 1 - DNA, 40 bp, synthetic construct
  source 1..40: mol_type = other DNA
aggtgacactatagaatatctccaacctcccttactacgc

SEQ ID NO: 2 - DNA, 37 bp, synthetic construct
  source 1..37: mol_type = other DNA
gtacgactcactatagggacggcttgatgcccacctt

SEQ ID NO: 3 - DNA, 38 bp, synthetic construct
  source 1..38: mol_type = other DNA
aggtgacactatagaataatccacaacaacaggcaccc

SEQ ID NO: 4 - DNA, 40 bp, synthetic construct
  source 1..40: mol_type = other DNA
gtacgactcactatagggacgacccgaagttgatgacgaa

SEQ ID NO: 5 - DNA, 38 bp, synthetic construct
  source 1..38: mol_type = other DNA
aggtgacactatagaataccttcaccttcccgccaacc

SEQ ID NO: 6 - DNA, 39 bp, synthetic construct
  source 1..39: mol_type = other DNA
gtacgactcactatagggaaacccgtccaccaggctcac

SEQ ID NO: 7 - DNA, 38 bp, synthetic construct
  source 1..38: mol_type = other DNA
aggtgacactatagaataactccttgcaggtgctgacc

SEQ ID NO: 8 - DNA, 40 bp, synthetic construct
  source 1..40: mol_type = other DNA
gtacgactcactatagggatgctggccctccaaagtagat

SEQ ID NO: 9 - DNA, 38 bp, synthetic construct
  source 1..38: mol_type = other DNA
aggtgacactatagaataaacttcagtgcttcgtggtg

SEQ ID NO: 10 - DNA, 37 bp, synthetic construct
  source 1..37: mol_type = other DNA
gtacgactcactatagggaggatgtcccatgttgagc

SEQ ID NO: 11 - DNA, 36 bp, synthetic construct
  source 1..36: mol_type = other DNA
aggtgacactatagaataaatctgaggtccagtccg

SEQ ID NO: 12 - DNA, 39 bp, synthetic construct
  source 1..39: mol_type = other DNA
gtacgactcactatagggacattaagaaggtggaaatcg

SEQ ID NO: 13 - DNA, 36 bp, synthetic construct
  source 1..36: mol_type = other DNA
aggtgacactatagaatatggaaggcgacggtgaag

SEQ ID NO: 14 - DNA, 37 bp, synthetic construct
  source 1..37: mol_type = other DNA
gtacgactcactatagggagcattggcaagggtggtt

SEQ ID NO: 15 - DNA, 39 bp, synthetic construct
  source 1..39: mol_type = other DNA
aggtgacactatagaatagaacctttcgcacgagatgag

SEQ ID NO: 16 - DNA, 43 bp, synthetic construct
  source 1..43: mol_type = other DNA
gtacgactcactatagggaggatacagcagccttcctttactt

SEQ ID NO: 17 - DNA, 38 bp, synthetic construct
  source 1..38: mol_type = other DNA
aggtgacactatagaatagcgacaacaatcccaaacag

SEQ ID NO: 18 - DNA, 39 bp, synthetic construct
  source 1..39: mol_type = other DNA
gtacgactcactatagggagagccactatcgtcaaatgc

SEQ ID NO: 19 - DNA, 39 bp, synthetic construct
  source 1..39: mol_type = other DNA
aggtgacactatagaatacaacgggatggagacggagca

SEQ ID NO: 20 - DNA, 39 bp, synthetic construct
  source 1..39: mol_type = other DNA
gtacgactcactatagggatcggaggcgatggcgaggat

SEQ ID NO: 21 - DNA, 37 bp, synthetic construct
  source 1..37: mol_type = other DNA
aggtgacactatagaatactgcctggctacttctccg

SEQ ID NO: 22 - DNA, 37 bp, synthetic construct
  source 1..37: mol_type = other DNA
gtacgactcactatagggatgccgttgcttcttccct

SEQ ID NO: 23 - DNA, 36 bp, synthetic construct
  source 1..36: mol_type = other DNA
aggtgacactatagaatacctcctccgccattcagt

SEQ ID NO: 24 - DNA, 40 bp, synthetic construct
  source 1..40: mol_type = other DNA
gtacgactcactatagggaactcctgctttgttgattcct

SEQ ID NO: 25 - DNA, 36 bp, synthetic construct
  source 1..36: mol_type = other DNA
aggtgacactatagaataggcagcaacagcctccta

SEQ ID NO: 26 - DNA, 37 bp, synthetic construct
  source 1..37: mol_type = other DNA
gtacgactcactatagggaacccgtcatccagcacct